European Patent Application EP 4 250 298 A2, published September 27, 2023. Title: Genetic test for liver copper accumulation in dogs. Applicant: Mars, Incorporated. Application EP. The sequence listing filed with the application follows.

SEQUENCE LISTING (246 sequences)

SEQ ID NO: 1 - DNA, 121 bp, Canis familiaris
  source 1..121: mol_type = genomic DNA
ctcagaactagataggctaataagtgataggccttgtgttttcctagagtgtgctttaaargtttcttaagctaaaaaattacattcgtgagaaaattgaaataaaaggaaaacagtcatg

SEQ ID NO: 2 - DNA, 121 bp, Canis familiaris
  source 1..121: mol_type = genomic DNA
tctcagatacttgatagccagcatttccccccattttcttccaagagcacgaaagcatagraatgatattacatctcgtatggtgaatgtgacacagccgtcagttgcgttagctctgctt

SEQ ID NO: 3 - DNA, 121 bp, Canis familiaris
  source 1..121: mol_type = genomic DNA
tattaccctgctctccagccactcctttaccttccattagcccacacctgctctacacacyattgctcatggaagccttgccacgtccagtcgccactctgaaatgccagcatccctccca

SEQ ID NO: 4 - DNA, 121 bp, Canis familiaris
  source 1..121: mol_type = genomic DNA
gacctgacagattatgtagactttgttttcaaagggagcacctgctggatatacaacatgrcactaaattgtgctccacatccttggcagaggtggggggcggggcacaaaggaagaaacc

SEQ ID NO: 5 - DNA, 121 bp, Canis familiaris
  source 1..121: mol_type = genomic DNA
gggcccagcaagtggcagaactgggaagaccccctcttcttccgcctggagcagtggtgtrgcagcacaccacaggagtctgaaagggtggggagtccaaacgggaacatatacctgagat

SEQ ID NO: 6 - DNA, 121 bp, Canis familiaris
  source 1..121: mol_type = genomic DNA
ggcaacagggacaggctgctgggccacacactcacccacactaggagacaagatcctccayatcctgggtctctatcagtcaatcacctagaccagtgggccagaggacagggtccagctg

SEQ ID NO: 7 - DNA, 121 bp, Canis familiaris
  source 1..121: mol_type = genomic DNA
gttgagagagatcatacagattcatgtggcaggtgcacactttttctacctcttacaacgyattctctctggccattccttctcctgggtcccaaagtcggagagcttagcgggagcctag

SEQ ID NO: 8 - DNA, 121 bp, Canis familiaris
  source 1..121: mol_type = genomic DNA
ataagttcacattttggtgtttcaagtggacatgaatggaggggagggccctgttcaatcyactaaagtgttttttcatcttgtttttgtggaaatcaaatcaagaagcagagttttatgt

SEQ ID NO: 9 - DNA, 121 bp, Canis familiaris
  source 1..121: mol_type = genomic DNA
actctcccgatgtgggcaccatatggtggaccactttctgtgtgagatgcctgctcttatygccatgtcctgtgaagacaccatgctggtggaagcatttgcctttgccctgggtgttgcc

SEQ ID NO: 10 - DNA, 121 bp, Canis familiaris
  source 1..121: mol_type = genomic DNA
aatctaagtagactgagtggtcaccttcagcgctcagacctgagcatacaaagcatggaargttactgtgattcagctgatgtaatggaatgaaataaatataagagtttggtaacctaat

SEQ ID NO: 11 - DNA, 121 bp, Canis familiaris
  source 1..121: mol_type = genomic DNA
tggagagtgctggcaggcaggggcaggcaaacaacaatagcaaagatctcttccacgcttytacttcctcaaaagtccaagccctcttaagatcgcattttcttagtgaccttcactctaa

SEQ ID NO: 12 - DNA, 121 bp, Canis familiaris
  source 1..121: mol_type = genomic DNA
ttctttgctaggccaagggcagagaatgcatgcccccccttacctcccagggcccaagagscatcctgagctgagtctatggctcctggtggggggcggctgtgggttgggggggcacaga

SEQ ID NO: 13 - DNA, 121 bp, Canis familiaris
  source 1..121: mol_type = genomic DNA
ggtgtcaccaatgccagcgagcaccagctggagggaacaggacacaggtcctccgtcctgygacactcggatctggggctttgcctccaaaacggagaccatgcctgtccatggttctacg

SEQ ID NO: 14 - DNA, 121 bp, Canis familiaris
  source 1..121: mol_type = genomic DNA
ctctagaacccttcaggtagactacattcactttctactacaacttcatcaccacaaccawctcccagtaaccccctttttttcttctcctttttttattttttccttctttttgctcgtc

SEQ ID NO: 15 - DNA, 121 bp, Canis familiaris
  source 1..121: mol_type = genomic DNA
tcccatgggttgaaggatatctggcagacggctccaactccagtaaagcctcaggcctcarccaggagttccccggggcttcattcccatcccagactttgcccagggctgatttgaaagt

SEQ ID NO: 16 - DNA, 121 bp, Canis familiaris
  source 1..121: mol_type = genomic DNA
tcttccttgcagattggatggctgtagcctcacctcacactgttgctgggatctgtccacrcttctgacctccagcaagagcctccgggagctaagcctgggcagcaatgacctgggagat

SEQ ID NO: 17 - DNA, 121 bp, Canis familiaris
  source 1..121: mol_type = genomic DNA
tattgctagtaaagccaaactttctattccacaattataaactcatggagatggtaattayagtgcattatttgtcaaattttattattttttcaaatcccaaagaaaatgtgatattcta

SEQ ID NO: 18 - DNA, 121 bp, Canis familiaris
  source 1..121: mol_type = genomic DNA
aagaacaaggatacaatctaagtgataatcatccagcatgtacttgtcctgttttcagatkatcagcttaagtcaagaggaatttttagtgcttacaaatatttcaagtgatttttccaga

SEQ ID NO: 19 - DNA, 121 bp, Canis familiaris
  source 1..121: mol_type = genomic DNA
tgaaggggtgctactcagggctcttcatttaaccttccaggatgttttcctatgtactcaytcttccttttggttgctccttcttcttgcatttctttatctctttacagaatcatccagg

SEQ ID NO: 20 - DNA, 121 bp, Canis familiaris
  source 1..121: mol_type = genomic DNA
acaaccctaaaatttcagtgattcagtacaacaaaggtttattataaccattcagggatcsaagttggtagaaacttcactacaatacctgcttccagtcaacaagacagaaaaagaaaaa

SEQ ID NO: 21 - DNA, 121 bp, Canis familiaris
  source 1..121: mol_type = genomic DNA
gcagggttgatatataactagtatgcattaggtagacacctattttgattactcactattktaatatcagcctggtagtaagaaccaaatctattatgtaaagtgcatagagaattgaaag

SEQ ID NO: 22 - DNA, 121 bp, Canis familiaris
  source 1..121: mol_type = genomic DNA
ctagctagccacccaactccccacatgcccagagtcatcgtttatcttttcacatcagcaytacattttggcttgcattcaaacattagcccattttttttccttttgttttatttataga

SEQ ID NO: 23 - DNA, 121 bp, Canis familiaris
  source 1..121: mol_type = genomic DNA
ttttctctttttccataaatgctctgggcttattttcattatctagtatttctcttctgargctaactcccaaagagttttgtgcatccttatttccatcacaaggtcaatgtacgagtta

SEQ ID NO: 24 - DNA, 121 bp, Canis familiaris
  source 1..121: mol_type = genomic DNA
gggcccaagggctgaggatctctgtaccttctgcttcttggcagcccaggctgggtagcakttcttggaagaggatttcccatgagttgttaacagaagggcgggcttccaggcgctgctt

SEQ ID NO: 25 - DNA, 121 bp, Canis familiaris
  source 1..121: mol_type = genomic DNA
catctttgcttggggcctggggtttttattgaggattgtgatctggtgtatgtgtctcctyaggcatccagaaaccattcagaacaagaacaagcgtccaggtatcctctgtaagtcactt

SEQ ID NO: 26 - DNA, 121 bp, Canis familiaris
  source 1..121: mol_type = genomic DNA
acaaaccctcagacccagatacacagtatcatgtggacacagacatgtaacaccaaaatgmccaacatcatgtgactacaggccctaagcaactaggtgtaacatcacttgggtatgggcc

SEQ ID NO: 27 - DNA, 121 bp, Canis familiaris
  source 1..121: mol_type = genomic DNA
aatgcagtaatacatgtagctaaacctaaccatcagagtctgttctatccttctacaaaartagggttggagctgagcacataggtagcatacatctagcaaaagtttttgccttcagatt

SEQ ID NO: 28 - DNA, 121 bp, Canis familiaris
  source 1..121: mol_type = genomic DNA
ttgtggggtcaggtgagttatggacccctccctactcttctgctatcttgccccctacagkggttgctattttgatgtaatcacaaaacgacctggcaataaaacctttttctaattaggg

SEQ ID NO: 29 - DNA, 121 bp, Canis familiaris
  source 1..121: mol_type = genomic DNA
gatgcaagctgggacagaataaggtactgggctgtgtcaagccccagtaagagaggagcaytgtagggtagttaggatggacttaatggagatgagtcctagggagccacactcagagtta

SEQ ID NO: 30 - DNA, 121 bp, Canis familiaris
  source 1..121: mol_type = genomic DNA
taaacacccccaatcactaccatcctcacacctaaggatacacaatgtgtctactttatgrtatgtctttactattcgttgcttatgaaattttattcattawctaaaacagggaaaaaag

SEQ ID NO: 31 - DNA, 121 bp, Canis familiaris
  source 1..121: mol_type = genomic DNA
tatagytggscaattaaatctcctattcttttgtctcaaaggatatttgaaattacatagytcttttctcatataaaacctaccatacaatcattagatgatccttcttagttaatttttt

SEQ ID NO: 32 - DNA, 121 bp, Canis familiaris
  source 1..121: mol_type = genomic DNA
gatgctgtgggccagtccagaacccacctgagagaaacaaacaggcctctttgccagcagrgcagcgtcagtgtcacccctgtgacatgtcagaacctccctgaaagttcatctaacctct

SEQ ID NO: 33 - DNA, 121 bp, Canis familiaris
  source 1..121: mol_type = genomic DNA
ggctcagaagaaaaatcagcccagttcacatccaatgtttccacacatctaatcgtcttgrgttcagaggtagatgtggtatcacttayatggacacatataacagctggcccccacctct

SEQ ID NO: 34 - DNA, 121 bp, Canis familiaris
  source 1..121: mol_type = genomic DNA
gtttcagttaattatagtccttactggatccgattgctgtggcgctaaaatgaaagaaggyagggtacctgggtggctcaggggttgagaatctgcttttgactcaggtcatgatcccagg

SEQ ID NO: 35 - DNA, 121 bp, Canis familiaris
  source 1..121: mol_type = genomic DNA
cagagtagcattattttctgctgtatgaggacacttttgttatatccacagtggacagaaractgggttttagaacatgctcaattgaaacaagactgagggctcacaaattcctgctcca

SEQ ID NO: 36 - DNA, 121 bp, Canis familiaris
  source 1..121: mol_type = genomic DNA
ttacttattcatctgagaccaaggccactgtggtgaacctacaaagccttacaaagcaggrccagaagggcacataaatcacttgactaacatttggtcaaaatagctcttgggctctttt

SEQ ID NO: 37 - DNA, 121 bp, Canis familiaris
  source 1..121: mol_type = genomic DNA
ataaaaataaaagagctattaataagaactcataaaatctacataaatatagtaacaggtyaatattcccagcatatttttacaaatcatctataaagagcatgagagcatatagggatta

SEQ ID NO: 38 - DNA, 121 bp, Canis familiaris
  source 1..121: mol_type = genomic DNA
gcaacaacctggtttgtgtgtgggaagctaatgcctccccaaatgcagcaaactctcctcytgattttagaaaagcagtttagttacaggcaaatgcatacatgcatgataaatactactc

SEQ ID NO: 39 - DNA, 121 bp, Canis familiaris
  source 1..121: mol_type = genomic DNA
gattttataaaacatgatgaccttggcatttatatagtagatattactactctgaaattcsaggaagtatgatcataaactcacacttaatctggtagaagtatggacaatgtatcaaagg

SEQ ID NO: 40 - DNA, 121 bp, Canis familiaris
  source 1..121: mol_type = genomic DNA
cttggttgagttaaaacatttgcccatgcaatttaatgcatgtccctgtggggttggaacygacgtacacccgagccaacagcctttcatggcagacgccatcaggcaggtgacccccacc

SEQ ID NO: 41 - DNA, 121 bp, Canis familiaris
  source 1..121: mol_type = genomic DNA
ccttccacacgctcaggttggcacggagggggtgtccttgcctgaggggtcctggcacagycatcagggcacacagctgataacccaagggagcagtaggcaagacctcatgggcgccggg

SEQ ID NO: 42 - DNA, 121 bp, Canis familiaris
  source 1..121: mol_type = genomic DNA
attctctttgctgtctcctgtatacagagataaaagcaagagttttccccttcaggtttcygaaacccagcttcctttagattttaaggggtattctgtgtacccatttcccaccttctgc

SEQ ID NO: 43 - DNA, 121 bp, Canis familiaris
  source 1..121: mol_type = genomic DNA
gcgggttgggacccccccttctgctgctcccacttcagagttgtggcgtcactaagatgasacctcatgtcgggaacctgagagtccctcgggagttgtgcagggactgtagccgacctat

SEQ ID NO: 44 - DNA, 121 bp, Canis familiaris
  source 1..121: mol_type = genomic DNA
acatatgcacagtgaatcgtggattgttgtgtttgatttcttacatgatacaataaaaggraagtagttgaagcaaaactttagtttaaaggaaacaatttctctatcataatgttcagtg

SEQ ID NO: 45 - DNA, 121 bp, Canis familiaris
  source 1..121: mol_type = genomic DNA
cccacagaccccaggtgctgaccacagcagccacttgggcccccaatgcaggagacacctygggaatgaaggggacaaggccagctcaggcacatcgtcagtgcacctgatgggaaggccg

SEQ ID NO: 46 - DNA, 121 bp, Canis familiaris
  source 1..121: mol_type = genomic DNA
atctgatcctagccaatggaaagcaatttgagataggaatcatatcttgttttggtttatrtgctttctttggagttttgcacatcatagataactgtaaatttgtagaataaatgtttga

SEQ ID NO: 47 - DNA, 121 bp, Canis familiaris
  source 1..121: mol_type = genomic DNA
gtcaatgccattaacctggcgaagctgctcgagcatccactgcgatctccgcacgaacgaygtggagccttcaaactgtttgaccttcgtgatggatgcttgtgtgggtttcttgtttgtc

SEQ ID NO: 48 - DNA, 121 bp, Canis familiaris
  source 1..121: mol_type = genomic DNA
actggttaataagacttcacagattttatccatcatgttgattatctgtatatgtattttytaccacttaggataaagttctgttatctgtaattgattccaaccagcatgtttgctccaa

SEQ ID NO: 49 - DNA, 121 bp, Canis familiaris
  source 1..121: mol_type = genomic DNA
cttcttctttcccattggattctttcatcaatcgtaggtagttcttaatgaagatctgtgrtaaagccattcatctattcattcaacaaatggcatcacagaaaagaaaaataacctttat

SEQ ID NO: 50 - DNA, 121 bp, Canis familiaris
  source 1..121: mol_type = genomic DNA
gggacacatttctggacagacctctgatcacactcacaggacagcaagaggaagctctggrtacaagtacagggaaaaaagaaagaaatggtcacagggaagctgccgcaggaaaaaggta

SEQ ID NO: 51 - DNA, 121 bp, Canis familiaris
  source 1..121: mol_type = genomic DNA
gggcagatcctcagtgagtattggctcatgttctccgagggaagtagagtcccagaagaargatgctaaggtgccaagattcctgagcctgtgtgtggtacagtcacagcagtactcctga

SEQ ID NO: 52 - DNA, 121 bp, Canis familiaris
  source 1..121: mol_type = genomic DNA
tcatctccatttgtaatagaaaccacatatatagagagattggattattaaccactaaaaygtagccactcaaggggagggggggaatgcatttggtttatttcccatgtcaaaacagaat

SEQ ID NO: 53 - DNA, 121 bp, Canis familiaris
  source 1..121: mol_type = genomic DNA
aacactgctaataaatatttataatggtttgaggaaaatatcaggtgtgagatgtcttcayatcatataatatatcataatatcctctaaaaaagctctaagcataggtctatggaactca

SEQ ID NO: 54 - DNA, 121 bp, Canis familiaris
  source 1..121: mol_type = genomic DNA
aagcaatccaggagtctttctccgggtagcaggctcgctttacaggttaaggctggatgaraaggaagaacctgagcttcaaattatcatctgagtagagctgatacccatggttacatta

SEQ ID NO: 55 - DNA, 121 bp, Canis familiaris
  source 1..121: mol_type = genomic DNA
gattttattctttactttgattttttttaagttttactatgatattcaatatgattgtggytcatgagattcctctttttagctgtatcattaactacagagcgttctcaaatatttttct

SEQ ID NO: 56 - DNA, 121 bp, Canis familiaris
  source 1..121: mol_type = genomic DNA
gtggccggagggggtgggccctactgtggcccagcttcacgtcccactggccaaacatcargatgcagacacccaggtcccttgtgctgcctgctgaggctaggagcagcgactggaaatg

SEQ ID NO: 57 - DNA, 121 bp, Canis familiaris
  source 1..121: mol_type = genomic DNA
gatgggagacctcatacacatgcaaagatcactattaaagactctcgagcaaagatcgaayggactgtggcaagctgccgcgcatgccaatcaacaaatgcctccgaccatggatctaacc

SEQ ID NO: 58 - DNA, 121 bp, Canis familiaris
  source 1..121: mol_type = genomic DNA
caacaaggtttttaaggttcttttcactaccttcttctttttgtacttgcttaggacaccygtatgtcttcacaatatcacctgaaagtcctttaggagatatactcaaaaaataaataaa

SEQ ID NO: 59 - DNA, 121 bp, Canis familiaris
  source 1..121: mol_type = genomic DNA
caacctgagctgaaggcagacactcaactgttgagctacccaggtgtaccaaacacatctrctcttaaccaagcttattctttgctatatttggcaaattgtggcatgtctacagtactca

SEQ ID NO: 60 - DNA, 121 bp, Canis familiaris
  source 1..121: mol_type = genomic DNA
attccccatgtttgaggaaatcacaggagccactaggaaatcaaccatttcccaaccaacytgatgatttcctgatccaaaggttctcccaggacaaatatgaggtagcctttcacactct

SEQ ID NO: 61 - DNA, 121 bp, Canis familiaris
  source 1..121: mol_type = genomic DNA
cagtcttgtaggagagtagattgactcacagaactggcaagattgggaatctgagcattgycacttgagtcttaaaacgtttacgattttatttctagtatttcaataagaaacacattct

SEQ ID NO: 62 - DNA, 121 bp, Canis familiaris
  source 1..121: mol_type = genomic DNA
gaatacattgccagaataatttcaagttctcaaatctcaactaataagattttcgttaaakaaggcattcaatcatcacttactgacaacccacaaaattaggcactgatgaaaaattagc

SEQ ID NO: 63 - DNA, 121 bp, Canis familiaris
  source 1..121: mol_type = genomic DNA
aagttaagatattcaagaaagagaagagagtgactgagctaaaaagaaaatcagatctctyccaggctttaaaataatctccacaatactgggcaatccatgtagtctccccagttccatt

SEQ ID NO: 64 - DNA, 121 bp, Canis familiaris
  source 1..121: mol_type = genomic DNA
ctcaaaaggaaaagcctgtggaaaggcaaagaggtatgtgaaagaggtaagttcaaaatgstgacatgaccagtgtacatagattacagggtacttggaggagcagtgagaaaggagtcca

SEQ ID NO: 65 - DNA, 121 bp, Canis familiaris
  source 1..121: mol_type = genomic DNA
ttctatgaaatagctaccattctggttggtatcttctgttgatttagatgatgaaggaagyataagaagtaaggcttatgagtttataaagctttagttaaagctttgattgtgacaaagc

SEQ ID NO: 66 - DNA, 121 bp, Canis familiaris
  source 1..121: mol_type = genomic DNA
agaggagaaaacacagctaaaaacttttttacagactggacaaaggtgcttacacttttcrtattgggcagaatgaggggatgaaaacaccagtggtctttttgaagccacacaaattcag

SEQ ID NO: 67 - DNA, 121 bp, Canis familiaris
  source 1..121: mol_type = genomic DNA
aggatgaatatttattaacagtaaatatacatttttattgttctatatactctaaagacarttgtagacagtaagatatatcaattttagaaacagaaataatgttaattgtataatatgg

SEQ ID NO: 68 - DNA, 121 bp, Canis familiaris
  source 1..121: mol_type = genomic DNA
cagggattcctaaagggtgacatggtatggtctaacacttcctcactgtccttttcccagmtgatataagaggaggaccagagagacacataaactgtctgagtctttagcattgtgataa

SEQ ID NO: 69 - DNA, 121 bp, Canis familiaris
  source 1..121: mol_type = genomic DNA
acactaatgggtagagaatacacgtccatcagtcatcaatgtaatctactaacagcctcasagtctggcagttttcagtgaaaagaggagtcatctccatttattcgatcaatcagttgac

SEQ ID NO: 70 - DNA, 121 bp, Canis familiaris; identical to SEQ ID NO: 3
  source 1..121: mol_type = genomic DNA

SEQ ID NO: 71 - DNA, 121 bp, Canis familiaris; identical to SEQ ID NO: 2
  source 1..121: mol_type = genomic DNA

SEQ ID NO: 72 - DNA, 121 bp, Canis familiaris
  source 1..121: mol_type = genomic DNA
acaggaaggagaactgagcatcaagagagttcagaacatgatcattgggtcagtttgtggstgcattaacttttccccaaaacagaaagcaacagagacttctgtaggtcagtcaacagtg

SEQ ID NO: 73 - DNA, 121 bp, Canis familiaris
  source 1..121: mol_type = genomic DNA
ttaccattactataacccaagttatagtatactataaccaagtccttaattgacttgatgyttgtgcagctgattttaaatctatttagaataatagtttacttgtgacaattcatattaa

SEQ ID NO: 74 - DNA, 121 bp, Canis familiaris
  source 1..121: mol_type = genomic DNA
ttggtcgactgactgattggttttactgtggaggaaagaaaagggaattttcccaaagagracagagagaaaacatggaattgagcaaagggagaatagagagacagggcagccactgaag

SEQ ID NO: 75 - DNA, 121 bp, Canis familiaris
  source 1..121: mol_type = genomic DNA
tgccttatcctccagctcctccctcaccatcttggaaactagctcaaatgtcactggtacktgtctttcttttgatctttctgaaagacaaacatgatcccatcacctctgcctttagaac

SEQ ID NO: 76 - DNA, 121 bp, Canis familiaris
  source 1..121: mol_type = genomic DNA
actcctaagtaaaagttaaattaacagatttgccatcaagtaccttgcccatttttcctayagatcgactttttactggatgatccccttgataataatcttgatctatgttttaattcca

SEQ ID NO: 77 - DNA, 121 bp, Canis familiaris
  source 1..121: mol_type = genomic DNA
ctggtgggcttgtcaggggcaggatgttgtgtggtgagcacagaattaaaactaggagctygaagcgcctggggggctcagttggttgacggactgccttcatctcaggtcatgatccctg

SEQ ID NO: 78 - DNA, 121 bp, Canis familiaris
  source 1..121: mol_type = genomic DNA
catacagcgaagagataaaaacacaggatgctgggctcacgaccatgaccggaaaaggacrgcgaggaaaagcaagtatgagcagcccaaagtcctttttccagcactggccataggagga

SEQ ID NO: 79 - DNA, 121 bp, Canis familiaris
  source 1..121: mol_type = genomic DNA
cagagatgaggaatcagactcctcgtcctctgcttctctacaatggctcatgttctccttycccctcagctgttgcattaacagaggtcaacccattcttctaaatttaaatctcccagaa

SEQ ID NO: 80 - DNA, 121 bp, Canis familiaris
  source 1..121: mol_type = genomic DNA
aatcaaacaagtgctagaacatagaacaagtggctcatcttttccccaaatgtctggatargaaaaaaaaaatctaaacaaatgctagatgttaagtatctgaaatgatcagcccatgaaa

SEQ ID NO: 81 - DNA, 121 bp, Canis familiaris
  source 1..121: mol_type = genomic DNA
tccataccagtccttgttgtctaccccgaacttcacctctctaggcacagacagctctaamtttcactcataggtatcttatgctgacctggcctgcctcctgttttgttttgttttgttt

SEQ ID NO: 82 - DNA, 121 bp, Canis familiaris
  source 1..121: mol_type = genomic DNA
caaaaaattccctgagcccagcatcaaggtacctggtttggagtgggtgggtcctcagaamgaatgggtgtggtgtacatttagcaagttatgtagcatgtgtctgtgtagtctcacctct

SEQ ID NO: 83 - DNA, 121 bp, Canis familiaris; identical to SEQ ID NO: 5
  source 1..121: mol_type = genomic DNA

SEQ ID NO: 84 - DNA, 121 bp, Canis familiaris
  source 1..121: mol_type = genomic DNA
atataatataacttatttaaaatatttgaagatatttctatagttatgctctaccatttgytattataagatttccaacagcttacttcttgtatgaaattaatttaccagcccctcacct

SEQ ID NO: 85 - DNA, 121 bp, Canis familiaris
  source 1..121: mol_type = genomic DNA
ccctattctataaacattccctctctggccatcctgtcaagtgggccctgacagtgtgccscagaagctccctagcctttgcccattccagctatggctagcctgccaccagccatacaca

SEQ ID NO: 86 - DNA, 121 bp, Canis familiaris
  source 1..121: mol_type = genomic DNA
cactgtgaggtctgaatggagacattcatgatagactccaggattttcccagctattaagycatgggccataaactggaacacttggaaacagtccataggttcatattaaagaatatgtt

SEQ ID NO: 87 - DNA, 121 bp, Canis familiaris
  source 1..121: mol_type = genomic DNA
gcaaaaggaacatgagttctgatcttctgtaaaggaggctaatttactaatggtcataacygtggcctgagggtcaagtttctaattaaacgtgcatcttggggyggactagaatactttc

SEQ ID NO: 88 - DNA, 121 bp, Canis familiaris
  source 1..121: mol_type = genomic DNA
caaggsccaggtaccctgaaggagtccgcttcacccaggcatgatgtgtttgacagtcttygtaattgatacagccattggcatcctcttgcggccaayatcagctccacttcaacctcgg

SEQ ID NO: 89 - DNA, 121 bp, Canis familiaris
  source 1..121: mol_type = genomic DNA
tgcaatgggttttgaaattagaggacatcacagcagagtagaatggtttggaacaggggartatgattaggattaatgagatgaaagaaaattctggctagagggctagaagagccatgga

SEQ ID NO: 90 - DNA, 121 bp, Canis familiaris; identical to SEQ ID NO: 1
  source 1..121: mol_type = genomic DNA

SEQ ID NO: 91 - DNA, 121 bp, Canis familiaris
  source 1..121: mol_type = genomic DNA
gatactttgggctctgggtgggagccagcagtggtggggcagggcaggagtccagcaaggygtctgggcatacatgtctgagagtaggaaaaccacaccattgcaccttgcctttgacttc

SEQ ID NO: 92 - DNA, 121 bp, Canis familiaris
  source 1..121: mol_type = genomic DNA
tcaaggatcagaaaaataaaagcaaagaaagaggcaaagaaagaagaaatgaaatacctartggcagaagtaggcagagaaataaaggctaaaagaaaatggcagaggattgtttgaaagg

SEQ ID NO: 93 - DNA, 121 bp, Canis familiaris
  source 1..121: mol_type = genomic DNA
tatgttatactattttagtatcttaataaatatgattagccaaaatagttttatcatcctsaaaagtgcagcatatattattttctattaaattcagaataggtataaactagaaagcatt

SEQ ID NO: 94 - DNA, 121 bp, Canis familiaris
  source 1..121: mol_type = genomic DNA
acagcagttctgaggatggactcgcagaggctcctgacaagcagaatgaccaggccgagcrgaaaggtcagtgctgccagtctagccagaagtgggggagagaggatgtaggagcagtact

SEQ ID NO: 95 - DNA, 121 bp, Canis familiaris
  source 1..121: mol_type = genomic DNA
actgtactcaaaaaagttctgtttgcctaaatgggatcagcctctaatggatgccagtgaygggaggctgttcatcatcccttcgggataattcagagcctaggcagaggcccagcgttca

SEQ ID NO: 96 - DNA, 121 bp, Canis familiaris
  source 1..121: mol_type = genomic DNA
tacaggccccaggaaggagccaccagatgcccaggactgggcccaggaatgatggaggctrtacagctggctgcctgcactggctgccgcccctgtcatccagtgtcacagagcagcacct

SEQ ID NO: 97 - DNA, 121 bp, Canis familiaris
  source 1..121: mol_type = genomic DNA
agacattgccaagaagtatccacaatgaacagtttgaaggggatccagaaaagcacagggyctacttccgctggatgagcagcagtgagaaccacagtcaggtaggtcttaaagcaaagtt

SEQ ID NO: 98 - DNA, 121 bp, Canis familiaris
  source 1..121: mol_type = genomic DNA
gctttgaaaaccaacaggaaatacatccaggaaagctatacaactgtggtgaaaggaaagraaaatctgctcttaaaaggttgtgtgcagactcacttgccccagaaaccagtgcgaaaac

SEQ ID NO: 99 - DNA, 121 bp, Canis familiaris
  source 1..121: mol_type = genomic DNA
gagatgtgtaaaatttaatagaaatgaaacttgccaaaacagacctctgtactcgtcagcrttctaagtccatctttctgtagcatgtaagtagaataatgttctattaatttcctctatg

SEQ ID NO: 100 - DNA, 121 bp, Canis familiaris
  source 1..121: mol_type = genomic DNA
gttctttctattctatcacacataccacccccctgcccacagtacccctttctgccatgtytcagactcctacacaagaggttctctctcctggcttccagttagacaggcaggtaaagct

SEQ ID NO: 101 - DNA, 121 bp, Canis familiaris
  source 1..121: mol_type = genomic DNA
taaaaaaatacaacagtagcattagaagacatgctaagcggctgtattagagaaggttagygctggcctgaagtttagaaaccttcccttctctttttttttttccttcccttctctttaa

SEQ ID NO: 102 - DNA, 121 bp, Canis familiaris
  source 1..121: mol_type = genomic DNA
tcaagagtactagagcatctataatcaatggtaaattggggaactagtgaaacaagtttayaggacaaataacataaataaggatttttttttaaatttggaaaattgtggaataatgata

SEQ ID NO: 103 - DNA, 121 bp, Canis familiaris
  source 1..121: mol_type = genomic DNA
agaattcaattttggggagccaggaaaccagattagttttccaaagggaagtgccatttgyatctatcccggtggggctgccaagaattccctggggtgggagacggcgcttctgtggatt

SEQ ID NO: 104 - DNA, 121 bp, Canis familiaris
  source 1..121: mol_type = genomic DNA
caccagagagccccgcaagatcatactgcacaagggctccactggcctgggcttcaacatygtaggaggagaggatggagaaggcatttttgtttccttcatcctggcaggaggcccagct

SEQ ID NO: 105 - DNA, 121 bp, Canis familiaris
  source 1..121: mol_type = genomic DNA
tggtgatgatttatcccccatgttcaagatttatcctccctgtctcaagaaatcatgtcaytacaggcatccttaaagtcacaagactgggaagtaaatactgatgaggtccaagacctgg

SEQ ID NO: 106 - DNA, 121 bp, Canis familiaris
  source 1..121: mol_type = genomic DNA
agcatagtgtacccacatataaggtcacatctgaggccagggagtcggggtcttgaagatkatgactgatcatgtgcttgaggatgatgatgatcatgtgcttttcctggctgtgcagttg

SEQ ID NO: 107 - DNA, 121 bp, Canis familiaris
  source 1..121: mol_type = genomic DNA
gtgtgtgtgtgtgtgtgtgtgtgtttaattctttgtgagaagcccctcattttgacctaartttggtagaggccccaggggatctgagaggagaacaaaaggataaaccatttgctgttca

SEQ ID NO: 108 - DNA, 121 bp, Canis familiaris
  source 1..121: mol_type = genomic DNA
ccaactttcactagcatcacagcccctatcaatctctgttcttttttctgtcagtaccatrtttgctcctactacatcyaatctgtgagctcacaggatgaggaccaacagctgccctgag

SEQ ID NO: 109 - DNA, 121 bp, Canis familiaris
  source 1..121: mol_type = genomic DNA
tgtcttacctctctctattcccttgtccatagtagtattaaatatatcttcctgaacacaratctgatccagtctctttttgtaattaaaagcctttgctagctttggtgatcacctccag

SEQ ID NO: 110 - DNA, 121 bp, Canis familiaris; identical to SEQ ID NO: 4
  source 1..121: mol_type = genomic DNA

SEQ ID NO: 111 - DNA, 121 bp, Canis familiaris
  source 1..121: mol_type = genomic DNA
cagaggaaaaggagaaggtcccacttaggggactggagaggagtgggggaacatcaccagmgccttcctgagccaggccccctgtggggagaagctctccccaggactgggtgcctttgaa

SEQ ID NO: 112 - DNA, 121 bp, Canis familiaris
  source 1..121: mol_type = genomic DNA
tcctccctctccccatccccattctcatgcaagtgtgctctctctctaaaacacccccccmcacacacacacacagacacaaccaaatttgggtctcaatgtcttgaccaaggaaaaggca

SEQ ID NO: 113 - DNA, 121 bp, Canis familiaris
  source 1..121: mol_type = genomic DNA
gagaagaaggaggagaaagaggaaaagtatatttgatggaatgaaaaacaagagttcaatytcactctggtctggggtgaccactattagtccttcaacatcttccttgaaggaattttaa

SEQ ID NO: 114 - DNA, 121 bp, Canis familiaris
  source 1..121: mol_type = genomic DNA
ctggaattctgtcagatcaacattcagagctccatcaaatctgagggaagcagtgatagargatacaatttgacctttcagtctattcaggttcatgtaggttaggcattcaatatcaaag

SEQ ID NO: 115 - DNA, 121 bp, Canis familiaris
  source 1..121: mol_type = genomic DNA
ccacatgtggttacaccactgtgttatccttccacctgtcccatcaacccacccgcacatrtcacagtgcctctgtcctcaaagaacactgtatccaacacctccacatcctctcagcatg

SEQ ID NO: 116 - DNA, 121 bp, Canis familiaris
  source 1..121: mol_type = genomic DNA
attcctatggtgggcgctgcacatttcctcccaggggaagggcaagggtcctgcatttctrtgctttccagggcctccgcaccaagagcaattgctaggtcacgcatgcccctgcacttcc

SEQ ID NO: 117 - DNA, 121 bp, Canis familiaris
  source 1..121: mol_type = genomic DNA
catgtcatcactaactaatttattaacaagagttttattctttgaaaaacaaaatcactcrcattactcagttgcttattccttgattcatatacaaatgactgataacatgagataaaaa

SEQ ID NO: 118 - DNA, 121 bp, Canis familiaris
  source 1..121: mol_type = genomic DNA
gatgatttagttgtttgaatgatctggcatataaatcttccaaatctgtgtccattggatygcttacagtttaatctttttatttcttcccagaatcacattttttcattatttatctttg

SEQ ID NO: 119 - DNA, 121 bp, Canis familiaris
  source 1..121: mol_type = genomic DNA
agttaaattctgtgaataactagaatccgttatactttttctgaaatgaagtctgtaggcwtttcaacagcaaaaggaattctgwttttyaaaactatacataatgcttcttaaaagccct

SEQ ID NO: 120 - DNA, 121 bp, Canis familiaris
  source 1..121: mol_type = genomic DNA
aatgccaactttaaaaacgcattcaaggttttcctctgtaaatgcattcctcattttggaygtgatgtaaaatcttattcagtgttttgtttttttttccccccacaggtctcaacaatta

SEQ ID NO: 121 - DNA, 121 bp, Canis familiaris
  source 1..121: mol_type = genomic DNA
ggtgggaccggccatcagcaggcgggccagcgccccacagatgttgtcacggacccgatcrtggcgctcccgtgccaggaggggcaacagaagccccagcagcttggggaagtatctggtt

SEQ ID NO: 122 - DNA, 121 bp, Canis familiaris
  source 1..121: mol_type = genomic DNA
aggggacttgtgctaatcactgggcaaattttatgaacttctgaattttaaagcaaaagaraaggtgaaagaatggaaagaaggtgtgagtgtttgaggaaaacttcttctttggggttga

SEQ ID NO: 123 - DNA, 121 bp, Canis familiaris
  source 1..121: mol_type = genomic DNA
tacacaagcaaggcagtatgccctgtctccttcccttgggccacctgcacttagacatggyaggttccagtgatgtgtctagtctctagcaagcagggcttgcttctgctctatccatcca

SEQ ID NO: 124 - DNA, 121 bp, Canis familiaris
  source 1..121: mol_type = genomic DNA
ctgtccttggtctggacctgctgtgaagaccaagtgcttcctgagatctctctgagtctartttccagagcagtgagtgagaaatgaaatgagccgaggattgccctccctcctatggact

SEQ ID NO: 125 - DNA, 121 bp, Canis familiaris
  source 1..121: mol_type = genomic DNA
taagccatcagcatgggctcctaggggtctgttcaactcccttgtggtgtcttactgctcragcaaaggaacagtctggtacagtgggagcaagagctgaggttggagagtggggacacag

SEQ ID NO: 126 - DNA, 121 bp, Canis familiaris
  source 1..121: mol_type = genomic DNA
gaggaggtggaagtgattaagtttaaaatttctggggtggtttctggcgacatgaagctgmgagctagaatgcctttcaatctcataatttctttaatttggtgattataccagagccaca

SEQ ID NO: 127 - DNA, 121 bp, Canis familiaris
  source 1..121: mol_type = genomic DNA
cctgacaaacactacctctgctcttcaaaagcaataagcatttattctgtgacacatttaratacaaagtcaattacaatagagtataagtacaatactagggaaagtacaaagtcatayg

SEQ ID NO: 128 - DNA, 121 bp, Canis familiaris
  source 1..121: mol_type = genomic DNA
gcatgatgaaatcagaaaaagtatgtaagtttctagaagaagctagatatatggtaacttwggtcaaatagaaccatgtagtgaaaagaatatgagttttcaagttcaataaaaaacaaaa

SEQ ID NO: 129 - DNA, 121 bp, Canis familiaris
  source 1..121: mol_type = genomic DNA
atgcataagtttccaaaagagttcaggattccaaaataaaagcttcactaaaagattcatmgcaaaagagtaatgaacaattaaagtcataggatatctaaaatgaaaaactgttagactg

SEQ ID NO: 130 - DNA, 121 bp, Canis familiaris
  source 1..121: mol_type = genomic DNA
agatggcttagttgtttctctttcctcctgaagtccacagcttagttacttggactctccraaataggatcgttggacatttgaggaaagctctagcatgaaagccatagactaaaaaaca

SEQ ID NO: 131 - DNA, 283 bp, Canis familiaris
  source 1..283: mol_type = genomic DNA
ctctcattttgtgtattgatttgaggactctgtcctttttgttctcttaggtgttttgtaaccatttttgtggttcttgccacaaaaggccttatgaagtcctgcatatgagtgatgtgcaggacaactttgactttctgacagccagtttttgtgttttgttmccttagttcccaagttcctatcttgtttacctcatgatcacattttaatatcaatgaaatttgtaggaaaacagcagaaggaaagatataaggttactattctctatggaccttggttg

SEQ ID NO: 132 - DNA, 223 bp, Canis familiaris
  source 1..223: mol_type = genomic DNA
ttgcagattatatgataaatatagttgtagcttcaaaaatgactataacgaacagaaaaaaattaacttatcaaaaacttttcaaatttccccatayacttaactaggtaggccacagagtatgatagtatgcaagttattaaaatctgttagcaaggcataacacatatatttctacttaatgaggtttctataatcaaggcttgtcaagtccattatgttc

SEQ ID NO: 133 - DNA, 157 bp, Canis familiaris
  source 1..157: mol_type = genomic DNA
tcagactgaatctaaagccacatatatttcctcagcagctgataacattagaaatcagaaagccactatyttagctggcaccgcaaatgtaaaagtaggctctaggacgccagtggaggcttcccatcctattgaaaatgcatctgttcctaggcca

SEQ ID NO: 134 - DNA, 179 bp, Canis familiaris
  source 1..179: mol_type = genomic DNA
tcttgtgcttgttctttatcaccattcattcagtacatccaaattttgaaatccttagagctctatagcctctatgtaggagaatgaratttcatcaaaaggaaatattttgagaatttaagtgatttttttatgatattttagctatagcagtcaccttgagccaaaagacattctac

SEQ ID NO: 135 - DNA, 191 bp, Canis familiaris
  source 1..191: mol_type = genomic DNA
aaaaatatactctctttcttacagaaacctctaataattcagattctggccatgaagttcaggaggattcttcaaaggaaaatgtatcatcaagtgctgcctcyactgaccacaacccaacacctactcatgatggcaaatcmcmtraactgtytawtytcsgattggrrawtmaaykgttraggaatgaa

SEQ ID NO: 136 - DNA, 244 bp, Canis familiaris
  source 1..244: mol_type = genomic DNA
tttgcccaagaaaaatgaagacctatgaccatggaaagacttgatacataatgctggagtactagtagtcagacccacccaagtcttttcacgtgttcattcagtatagatgcggcacacgttggctgagtccctccgktgtgtcaggaactgttttaggtattggggatgaagtagggaacactgatttagsttctgtttattcatgtctcactttgtaggaattycmhtamatagaaraada

SEQ ID NO: 137 - DNA, 251 bp, Canis familiaris
  source 1..251: mol_type = genomic DNA
tctcagtactcacaggtacttacaaatacaacactaagaggtttcacaaaacagtactcttacatagcacatgctgtactctctgttccattctattttattactattttaaaatatggattgtgatytgccaakttgattctctggcccattaatagtttgaaaatctcttctgtaggagtataggaattaccacagagttttgagaaattgatgaatgccacgctttacctgtgggaacgtagattcta

SEQ ID NO: 138 - DNA, 191 bp, Canis familiaris
  source 1..191: mol_type = genomic DNA
cagatgatgagtctggagctggtgatctgggctggagataatgaacctgggagtcatcagctttggagaaagggtgtctggcctcactcttgctwgcacagaaagaaagtgctcattagtgtcaactctcagcaacacttggtatttgtaaactttaatttttgctgacttcatggagaaataatgttttt

SEQ ID NO: 139 - DNA, 206 bp, Canis familiaris
  source 1..206: mol_type = genomic DNA
taatgatacagaaatgaatttggcaggaatgtatggaaaagtccgaaaagctgctagttcaattgaccagtttaggtaagcaagtgcagtactggtgaggaatggkgcatcggctccttctgtgctattttccggtggctccagtcacagccccatcaagcagagctgatacctaaagtgacatttaccctacttcctctctcaat

SEQ ID NO: 140 - DNA, 186 bp, Canis familiaris
  source 1..186: mol_type = genomic DNA
catcacttaaaatcatctcagcaagtgttgttgaagatgattttttataaagtatattccaatcttattctatacttcagaagcttggaattctyatttgctttgctggattgaaaaagtctggaagtaattagaatgacttctcatactcccaccttgaattctcctaatatcaaaggctgggag

SEQ ID NO: 141 - DNA, 171 bp, Canis familiaris
  misc_feature 169: note = n is a, c, g, or t
  source 1..171: mol_type = genomic DNA
atatggagaaatgagctcttatacactttcagtggacatgtaaactgttattgtctttttggagagcatttggcaggatctatcaaagtrcacacatcatttgattgagcaattccacttccagccatattctggacataatttacaagtataaaaagatgcatgtttnga

SEQ ID NO: 142 - DNA, 213 bp, Canis familiaris
  source 1..213: mol_type = genomic DNA
aaatattgaaagtgctttatctacactccaatatgtaagcagcatagtagtttctttagagaatagatctgccatagtaaagtacaatgcaagcttagtcaytccagaaaccctgagaaaagcaatagaggccatatcaccaggacaatacagagttagtattgctagtgaagttgagagtacctcaaactctccctccagctcacctcttca

SEQ ID NO: 143 - DNA, 125 bp, Canis familiaris
  source 1..125: mol_type = genomic DNA
ttaaaataactacttgcagtgatttctttcccccagtataaaatgtcagttttgtctcaatccacccycttcaccttaaaaagaaaaagaaagtattagttttcagtgtcatttgccttaaaatg

SEQ ID NO: 144 - DNA, 201 bp, Canis familiaris
  source 1..201: mol_type = genomic DNA
gagaggtacgaggcccaggcgcagggccgcatgaagcccctgacggcgtcccaggtcagcgtgcacattggcatggatgaccggcggtgggactccccgcrggccacgccctgggaccaggtcagccgtgtcagccaggtgtctctgtcctccctgaagtccgacaagctgtcccgacacagcgccgcggccgacgacggc

SEQ ID NO: 145 - DNA, 201 bp, Canis familiaris
  source 1..201: mol_type = genomic DNA
ggtctgcatttggaacacctgcccagtggttgttaaatttaacccctgctaagagaatgagaggacagcacccctggagagacagaatccaggtgcttgcrgttctccatacgtgcactgcagcaggatccccagagttcaagcaccaagttctgcagggagattgcaggtcgcagcagaggtgctgttgtgctcgttctg

SEQ ID NO: 146 - DNA, 201 bp, Canis familiaris
  misc_feature 8: note = n is a, c, g, or t
  misc_feature 65: note = n is a, c, g, or t
  misc_feature 148: note = n is a, c, g, or t
  misc_feature 152: note = n is a, c, g, or t
  misc_feature 181: note = n is a, c, g, or t
  source 1..201: mol_type = genomic DNA
cggggctngatctcacgaccctgacatagtgacctgagccaaaaccaagagttggacgctcaatngactgagcctcccgggagccccaaagtcaagagacrctacagatgcgttgggcacaatgacaggggaggaagctgaggtctgntggnggaggttctgcacctcccagcaggacccngcacacagcaggtgcctgct

SEQ ID NO: 147 - DNA, 201 bp, Canis familiaris
  source 1..201: mol_type = genomic DNA
ggggagtccggcatggccccctgtcagccctgtcccctcagggtgtcttggccgggttgctccctgacaagctctccctcctctctcttcaggttcagccygaatctgacaccatgcccctagggaagagcagcgagctttggaagcagggagaagacctataggaggccgagggcctggggatgcccagctgtctggggc

SEQ ID NO: 148 - DNA, 201 bp, Canis familiaris
  source 1..201: mol_type = genomic DNA
ccttcagagagaacccaggacaattactaaactaccgtgccctggaagatgttttgtgactcctcactccctctgccttgcttattggccattattttttkatccctctctcttctaccattattaatcaaacacaacaaacaaaacacttctaacaaggatattaggtttgtatacattttttttaaaaacagcaactta

SEQ ID NO: 149 - DNA, 201 bp, Canis familiaris
  source 1..201: mol_type = genomic DNA
acttcctgattgctactgtctggacactaggttttgcgatttgttctccccttccagtgtttcacagtctggtggaacttcaggaaacatttgactccgcrttgctgagcagcaggtatttatgtgttgagtcgtggccatctgattcgtacagaatcgcttttactatctctttattgctagtccagtatattcttccct

SEQ ID NO: 150 - DNA, 201 bp, Canis familiaris
  source 1..201: mol_type = genomic DNA
cagggaacattttcaaagatgtagaaaatcccaagacatgttaacatagggaatgcatgtaaagatgcaatcaaaagcctttgaaatgacaaccacttatrtaagacctagcaatgtgcacttccaaacattaactaaaagttctatctcccccctctgggttccttaaacattacacctctctgcctatcaaagcaccta

SEQ ID NO: 151 - DNA, 201 bp, Canis familiaris
  source 1..201: mol_type = genomic DNA
ttcctcataggaaatttggccttctctgatattttggttgtgctgttttgctcaccttttacactgacctctgtcctgctggatcagtggatgtttggcaragtcatgtgtcacattatgccttttcttcaatgtgtgtcagttctggtttcaactttaattctaatatcaattgccattgtcaggtatcatatgatcaag

SEQ ID NO: 152 - DNA, 201 bp, Canis familiaris
  source 1..201: mol_type = genomic DNA
atccagaagaagtctgctaggggtaactatcttttcgctctctgtttatgccaacatttcacaaaagcttgtctcccgtgacttaaatagatacacccagmgtgtatgttggggatttttgcaagtatccttaggaggccctacgtcgtaaggcacagtcataagacctcgcgtccctattccctcatctgtaaaatggtg

SEQ ID NO: 153 - DNA, 201 bp, Canis familiaris
  source 1..201: mol_type = genomic DNA
caaggtctgtggatgtgcttactccgtcctcaccacaaacaccgatgtctcggacacactcagtgagcccaggttaggaagccaggattgcagggccaagrgtataaggaggtgtcctgggagcctcaaaagaaaaatacaaaagtatgaagactcagaataaattcttacaaatcttgctgtgtcttcccacagatggca

SEQ ID NO: 154 - DNA, 201 bp, Canis familiaris
  source 1..201: mol_type = genomic DNA
gaaaggccgtttcctacctcggccccaagtagtgagggcctggaccctgagcccatgatggaccaaagggagcaggtgggtgaggccccagcccttggacrgaatatttcattagctaatgcaaatcatgagttcagggaatcctcacagccccctgagaatacgcagagcactgtgttatgtctcccagggtccctttta

SEQ ID NO: 155 - DNA, 201 bp, Canis familiaris
  misc_feature 56: note = n is a, c, g, or t
  misc_feature 100: note = n is a, c, g, or t
  misc_feature 130: note = n is a, c, g, or t
  source 1..201: mol_type = genomic DNA
aaagtatcagcacactgatgcagccagcctagctgaagatggagttgttgaagcanaggtgttcatgatccctccccagtgacctgcgattttttttttnwaatcttattcgcccattttattaaatccncaaattcaaatctgtttgtctcacttgctgagatttcttttgtctttctctttcattcattcttacagttg

SEQ ID NO: 156 - DNA, 201 bp, Canis familiaris
  source 1..201: mol_type = genomic DNA
  variation 101: note = n is cytosine or there is no nucleotide present
aagaaaaagaaaaacccagccatcaagggtgtgcatgtctgtgaaagctccagacaggatgatcgaggttgtttgcaacgacagtctagagaagaaggtgngcgttaagtgcaacactgatgacaccatcggggaccttaagaagctgattgcagcccagactggcacctgttggaacaagaccatcctgaagaagtggta

SEQ ID NO: 157 - DNA, 201 bp, Canis familiaris
  source 1..201: mol_type = genomic DNA
gcctagcattattcctgacatgtgttaggtcctcaacaaatagtagctaatatactttctggatttctttctttttggctaagtagaagagctggtgctgycatccttatagtctgtatagtaggatttcttttctttccttttcttttttaaagattttacttatttactcatgagagacacagactgagagagagaggc

SEQ ID NO: 158 - DNA, 201 bp, Canis familiaris
  source 1..201: mol_type = genomic DNA
agagagaggagaagcaggctctatgcaggaagcccgatgtgggactcgatcccaggtctccaggatcatgccctgagccaaaggcaagacgctcaaccacwtagccacccaggcgtcccttttaccttagtttttgtcctaaagcttcatataaatggaatcatgtagtatgtatgtgtgtacactctcttttctgacttc

SEQ ID NO: 159 - DNA, 237 bp, Canis familiaris
  source 1..237: mol_type = genomic DNA
tgcctctccactactcactcttctcttgaaagattatttcctgcttaaactggcccgtgacttcctgctgccagaaccatggaatggcctcctgagggaggctccctatgctgctcccatyagcagatattgcagcgtcacagtataactcagtggcttgaaatgatggctatttatcattgctcagtaatttgagtggctcgaagaggatagaatttcatttctttctcagataat

SEQ ID NO: 160 - DNA, 237 bp, Canis familiaris
  source 1..237: mol_type = genomic DNA
tgtacagctgactccctgagaaaggacatcctgggtcacctttcaagtatttcctggcatggaaaccccatatcttcaaacacaaaaatcagaaaatcacagtccttatctgtttgggccyatttataggagagtctttttattgcctggaattgtatatttttacatttcttagatttctacaaaataatatttgtgccttctttcaagtataatattatttattaaagttgcttt

SEQ ID NO: 161 - DNA, 237 bp, Canis familiaris
  source 1..237: mol_type = genomic DNA
attaatacattcttagtgtcttctttaaaaatgcaacttccatgctttataaaataccaacaaatgctttacatctttatgatggtaattttggatcaatactggaggattttaaaaaaayctctgcttcccctgcttgtgtggtctctcacgcgctctcattctcactctgtcaaataaataaacaaaatctttccaaaaagacaaagtccttgtgaaaactgagaaggcctgtga

SEQ ID NO: 162 - DNA, 237 bp, Canis familiaris
  source 1..237: mol_type = genomic DNA
atttgtactttcttttcacttctcctgcgtggtgcgtatctctccagtctgtgttctttaggcatacattgctgtatgtgctttaaatagaatcctaccttatatactgcttaataacctrtgaccataagatcaggttccatgtcttcaaagattctcctcatcattttcacgggtataggcatagattacaattgatccattccccactttgcacatttagattgttttcacttt

SEQ ID NO: 163 - DNA, 237 bp, Canis familiaris
  source 1..237: mol_type = genomic DNA
tgcaatgactctgtttacaaataaggtcacaatctcaggtaccagagcttagggcttcaacctgtcttgggggagggtgggcaggataccattcagtccataacagcagaagatcccggtygtcctcacagtatggtgggcagtggccagccctccggactttcacctccagggggcaggcggagaagctaaaggggggtctcatggcctcccagctcctccctttgcccctgcaat

SEQ ID NO: 164 - DNA, 237 bp, Canis familiaris
  source 1..237: mol_type = genomic DNA
acccacgcccagcatctaagaggccaacccctccctgctgtgggctcctgggcttctcaacccccaaggaggggactgcagtccagcgtgccgacagctgcctccaccccaaagggggccratggctggtgagtggagactgagtgcatgaccgacttttttagccaagactttttcttaattgttagagatggcaaactcaagcaaatgggaaactcatccgctcaagtaaccagc

SEQ ID NO: 165 - DNA, 237 bp, Canis familiaris
  source 1..237: mol_type = genomic DNA
gcctcgtgggacagctttctagcactttcccctttttaagagattgactgcaatttctataataacatcacattagctagaaattaatgtcctcattaagacagcaattaggcacattagygcggcaataaaagagaagcttatgaaataattgctggttccgaaatgcctttaatttagtgttttatattgcgccatgttattaattttttccctcggcagaagataataagagaa

SEQ ID NO: 166 - DNA, 237 bp, Canis familiaris
  source 1..237: mol_type = genomic DNA
cataaatgccccccccacctctgtgtctgtgcagaaaccaaaagtcttgggcttctatgatccccagtgagtgctaggagcaggaccgcaatcacagcagcacatcctagaaaggacttargagccagatactaccatcctattcactcaggtaatcctcacagtaaaccgcaatggcataaaaaatattacctccagggcccaacggacggactcttgatctcagggttgtgagtt

SEQ ID NO: 167 - DNA, 237 bp, Canis familiaris
  source 1..237: mol_type = genomic DNA
atgagatatgtctgctcagccactgtctggggccttgtaattgaagccttataattagcatgaagtcaccagcttggtcctgctgaaagggcacagggtggggtgtgaaaggaggatggcyaagggctcgtccacaggaaacattttctaaacactagagaggaggcagccaaagagctcccttcctcatcgcccatggaccccactgctatgctggcaattccccttttggttaat

SEQ ID NO: 168 - DNA, 237 bp, Canis familiaris
  source 1..237: mol_type = genomic DNA
ttcctgtgcagagggacacgtgaaggccctaggtcctcctgggagaaaagatttccctcctaatgatccagggactaggatttcattctgaaatggaatggagaatggcaggtgtggcttkctggggattgagaaccacaggccccaggagattcaggaaaggacagtaatgccctgctgctcaggccccggtggaggaatcatatcctcagctcagcaacaccacccgccccccta

SEQ ID NO: 169 - DNA, 237 bp, Canis familiaris
  source 1..237: mol_type = genomic DNA
acatcggctaaacaaaaacaggagaatcccattataagacggttcctgtagtacagatgtgtctgggtgaagcctgggttgtatcgtggccccatgtagagccagcctgggcagagagctrgtctacccactaagcaactgcaagaggcaaagtgcagcattgatgtcacgaggtccagcatcaactaggaccatccccatccatgtgagcaggctcacacgtggaatcgcagtgga

SEQ ID NO: 170 - DNA, 237 bp, Canis familiaris
  source 1..237: mol_type = genomic DNA
ccgtgcttcacaggcgagaatctgaatgaccgtgatgccaccacatgtcaccatccccttttccactgggaaaggggtccttgttgccttccagctccagaattgcatcctcacaatttcrgaggcccttcctcctgctaagctctgtgcttttccagaaagtagagcataagacaagggcttatatgcaagtatattttttggaaaatatgatcccagagagcaggagtgagaact

SEQ ID NO: 171 - DNA, 237 bp, Canis familiaris
  source 1..237: mol_type = genomic DNA
actccatgaaatggtttattttatcctatgaatcgatgtggagaacaaaggcaaaagaaatatagaaaaatattaaatttccttacaatgtacagcccattgataatattttagacagtgwgagtgatcttgcttatggagctcaactgcctcaatgttaatccttagctaaaggcaaaagacaatcttagtttgacattagcctgaccgccttatgctatccctaacccccgtccc

SEQ ID NO: 172 - DNA, 237 bp, Canis familiaris
  source 1..237: mol_type = genomic DNA
aatccaaatactccatgaaatggtttattttatcctatgaatcgatgtggagaacaaaggcaaaagaaatatagaaaaatattaaatttccttacaatgtacagcccattgataatatttkagacagtgtgagtgatcttgcttatggagctcaactgcctcaatgttaatccttagctaaaggcaaaagacaatcttagtttgacattagcctgaccgccttatgctatccctaac

SEQ ID NO: 173 - DNA, 237 bp, Canis familiaris
  source 1..237: mol_type = genomic DNA
aggaaaaatatgcttgcttttgaaggaatcaatttgtggtttcttttaatgagttatcaaactattaataagcattaattatttattgtgtaaggcaaagtgcttcttaataggtattctktccttaacttagaacattcacagattcccaatagcctctagtgcagaagaagtctgccgctcttctttcctcctttcactagtctctcctatatctgtgatacctccaatcatagc

SEQ ID NO: 174 - DNA, 237 bp, Canis familiaris
  source 1..237: mol_type = genomic DNA
cttccatgttctgtctccctttctgatatttcctactcattccagaaaatattcttaatgaagcctctgatacggtcttgaggatcctcagagaccatatgtcagtctgtcaatgaagcaraaatcaagatgtttggatccctagtagatatgtaatcaaaatgccatgggaatacagagaaggggagtcatttgtatcagttagtgttaaaaattattatcacgctcttgatatta

SEQ ID NO: 175 - DNA, 237 bp, Canis familiaris
  source 1..237: mol_type = genomic DNA
gagaatactgaagacgtaatgaagttgagttccacctttataataattccgttttaccctaaaggggaatattcaaaaatgtgacatcgctctaccagaccaccttgcgactgctctaaamgattggcaggggcaagaacttgtgtcactgataggcgggattttttagtcctctctgcaaatcattaagaaaatgttccaacgcaacaaaacaaaatatggtggcgatccctgaac

SEQ ID NO: 176 - DNA, 237 bp, Canis familiaris
  source 1..237: mol_type = genomic DNA
acctgataacaccgcctcagtggagaacgagttggcacttcaggacagatttccctgccagagcctattcctgtttgacactttcatttgaagaaacccactcatggtttcttctctccarggtttaaaaccgagatcaagtatatctctttaataatgtcacattccaaagaatgactccgataaggggattgttcaagggcttgggtattcacataagggctatcatgcggggag

SEQ ID NO: 177 - DNA, 236 bp, Canis familiaris
  source 1..236: mol_type = genomic DNA
tcctctagatctgacctacatttcaaaaatatatgagtgggctataaccaggaatgtcttctcttgctgccattattcacactgcattttctgaagttgtttttttttttttttttttttycccctcggtgactttaatggccattgagggaactgtagacattgggagtctttatacagccctagtgaaatggcgagtgttatcaatagggtggctgaatggtacggctctgggc

SEQ ID NO: 178 - DNA, 237 bp, Canis familiaris
  source 1..237: mol_type = genomic DNA
catctgtgacccttggattcaaaccaagtaggatgcaaacctcagaacttctggcatttcggatgcactgatctctgccagccccttgccctcttctaatgggatagaagctgatgatgtragacaccgcgtgcaccatctgcccaagacgtcccagttgatgccactcatcctggtttgtgcaaaaaattctctatttgccctaattccaccgctcagcaactggaaggacctgag

SEQ ID NO: 179 - DNA, 237 bp, Canis familiaris
  source 1..237: mol_type = genomic DNA
tcacaatggcttttttttttttaagatttaacaggaattttgtgatcctttatatgatatgtttcaatgaagccttttgggaaaggttcttaatgtgaaagaattttcacagagaatatcrgaaataaatgtgcaaaagggagtcgttttaggattagagatatgcatggaagagggaaaaagcctacttatattactagaaaataattttcaatttagaagttatactgaactatt

SEQ ID NO: 180 - DNA, 237 bp, Canis familiaris
  source 1..237: mol_type = genomic DNA
cccatttttttaggattgataaactgatcatctaacagatattatatacaaaagtcagagaagacacaatagccaaccctgtgtgtaaggaaaatgacagagttggttaaagagaaaagaraaaggaggtacacagagagatgtagaggtcacattaaaaatgaacgttgtccatgtctatgaaagatggaaggtaattctatgcctataaggtatgttataagttaaattaattgt

SEQ ID NO: 181 - DNA, 237 bp, Canis familiaris
  source 1..237: mol_type = genomic DNA
aacaaacctaccaaacaggacaaaccagtccggattatataatatgtaaatatgccagggagctggggagcatacttgtgggaggataagctggagcaatggttaaatgagctcaatcctyactatacttgaaggtagtagcctcttcattcacactccatggctagccctttgtaactaaaatatggaaaacacaaccaatgaagaagttacatgtatccctaaaaataccaccta

SEQ ID NO: 182 - DNA, 121 bp, Canis familiaris
  source 1..121: mol_type = genomic DNA
cccttggcgttctaaagtccagccccctctcttcgcattctgtgctttctcctgtgtggcrgtctctgtgctttatctgcacataaacacttcacaaatttccgttccagcttagttctct

SEQ ID NO: 183 - DNA, 237 bp, Canis familiaris
  source 1..237: mol_type = genomic DNA
ttaagtttagaaaaaacaaattcaagaacaagctttttatatttaacatcgatgaatcagaagatacggggttttttaaattattaaactaaaattattaaactggtcctgtttggtataragttatcttaattatgctaatctggaatcttaaagcatttttaaactaatattttaagaaaccaagttttagatttattccaaccttgggctagaaaaggatgacctttgtgggcc

SEQ ID NO: 184 - DNA, 237 bp, Canis familiaris
  source 1..237: mol_type = genomic DNA
tgagccacccaggtgccccaaaacatgattagtcttgaaacaaagtgtatcacaataatgattcaattagatgaataaaatgtagtttttgagaatggtaaacactatgtaagagtaaagytagcctatttgatcagtaaacctatttaagtttagaaaaaacaaattcaagaacaagctttttatatttaacatcgatgaatcagaagatacggggttttttaaattattaaacta

SEQ ID NO: 185 - DNA, 237 bp, Canis familiaris
  source 1..237: mol_type = genomic DNA
agatgtcatgctatgatatatttaaataagttacagacatgtataatttccatggtatgttttacattcatataaaaattaactattcataaaatataataaaatgtagtgtttttcttaytgagcttcagtgatcataatttgtatattaacttaatgaccagaaataattaagtaaagctagttaaattcttgggatgttatggattatgttatttggttggctgttcatgataa

SEQ ID NO: 186 - DNA, 120 bp, Canis familiaris
  source 1..120: mol_type = genomic DNA
tgttttgaatttaaggtgtttttccaggctgagaagaaacgtgagctcttggaaattatrattaacgtatctaatgcatataccctagagggcaaggaaatttctattcattccctgtat

SEQ ID NO: 187 - DNA, 237 bp, Canis familiaris
  source 1..237: mol_type = genomic DNA
cccccaggatctgtcagtaatccctgactgcctgcagaccacatggggagagggatccattcctatgacagagaatttatactggcttgtgagctgaacagatacctcagaagatgttcayctgtgagacagagagacatggtgacaaatacaagtgtcagccaacagcagcaccaagtccaggaatggctgcctgagctggatggaacctcactatccagagccatccataggccg

SEQ ID NO: 188 - DNA, 121 bp, Canis familiaris
  source 1..121: mol_type = genomic DNA
agagccaacgctggatctcagggagaatctagaaggccagctgaccagaaaaccaactggrcagacagaagctgggagcagcgcctgtggaggcaggcacgagaggccccggtgcagccgc

SEQ ID NO: 189 - DNA, 237 bp, Canis familiaris
  source 1..237: mol_type = genomic DNA
ctgggtggctgttggagagagtgtgttgtgttgttcccagggttagtcctaggaatggtagagcctgtcaagttctccctgaaagtcacgtcactccccacttcagcaggcccagcctgtsttgtatccctgcagcactgcctcaggatccttgctctgcagtgatcagagtcatctgataagcctgtccctgtctaggctgatattaatttcaggttgtcaccctctatgcctctt

SEQ ID NO: 190 - DNA, 237 bp, Canis familiaris
  source 1..237: mol_type = genomic DNA
ggccttatgaagacttctctgatctgttgatctgatgtacccagattctgaatccctaattagactcaattaggacactcctggaggtgactactgctttcttagactttgtcactcaaayatctaatacattcgactttgacccatggatttattgagttcctcttgcacacccagttcagtagatgtggtccactattttggtgcatcgactgctctagaatttagcttttggaa

SEQ ID NO: 191 - DNA, 237 bp, Canis familiaris
  source 1..237: mol_type = genomic DNA
atgacacatgcaagtgctcaataacgttagacactgtactgttaattaaaggtctatcgcccctttaaacaaaatgtccagaatgttcatgttcaccaaaagtgaaaggcattcatgtctmtgtttctgttgagttcactgtcacctttgtgcctagaaaggagaagacacactggtttttcctcctctagagaagtgcagatttgtataggtgaggagtatacataggttgtgggc

SEQ ID NO: 192 - DNA, 237 bp, Canis familiaris
  source 1..237: mol_type = genomic DNA
ctttgggaatgaggcctgtcccgctagcctgcttcatttactctcatgattcttggcaaagttcttataagtcacgttcaaattatcaggcttcattcctagtctgagcagacttgtcccrtctcccagcctgtggatgttcaagaagcgcaacttggttttatgtttattaatcaaaagccctttagcctctgatgaacctctgagggtggctttaaagccccgcgcctgctctga

SEQ ID NO: 193 - DNA, 237 bp, Canis familiaris
  source 1..237: mol_type = genomic DNA
aaagaaaaaagtaagggtcaaaacactagcaaaattaaattaaaaaaataagaaaaacaagtcacactttttttttttttttggtcatttgggaaaagcacaatattttgcttgattactyttcctcacttttcaactagtaatatagattgcatgaaaaataaacaaaacaagtaaactttaaatgtttgctggtgtagaggtgaataagaacaatccatggattttgcaatcaca

SEQ ID NO: 194 - DNA, 237 bp, Canis familiaris
  source 1..237: mol_type = genomic DNA
tctagctccagtctcctttattcagtgccaccttcatttttccattccagccaaattagtgttttcattctctcaagcattttcatctatgtacttcctgaaccctcttcatggaagacaycctctactcttcagcatattactatcccagcatcccttaccctgatagtttaacttgattctttatctacctgattcagtaatatttctctattcttatcatattcagcaatgttc

SEQ ID NO: 195 - DNA, 237 bp, Canis familiaris
  source 1..237: mol_type = genomic DNA
tcccctactgaaaacaaattcccccatcttcaccctaccatggggattttacatttgttaccagatttggggcaaactcatcctattttcccttcagtgtggagaagagattttggaaagyagaccatgcaaatctctaagctcacaataaactgaattggagaggcataaaacctgacaggaaaaaaaggtgtgaacttgatctttagcttgctgttctggtttaataggtttctg

SEQ ID NO: 196 - DNA, 237 bp, Canis familiaris
  source 1..237: mol_type = genomic DNA
aagggtgaactgacttttagtcagaatgtttatttttaacagattataaaatagccacctatttagatggataaatgtattgtgattatggtgttgtttataaaaagaattttcaggattktccacaaaacttaatgttagtattagttattaagagtacaatggaatatcattcagccatataaaagaatgaaatcttgctatttgcaatgacatagatggagctagagagtataa

SEQ ID NO: 197 - DNA, 237 bp, Canis familiaris
  source 1..237: mol_type = genomic DNA
atgagtttgcaattctagccggtgcatgaggacttctccctttcccgagccctcccggaaagtttggccagatccccagcccaaatggcagcatgtgctcgggaagatgattaatgttagygcgaggctccagagaatctctcagggcccttttgtttattaaatagaaaaattcatgtttaaatataatgtcaaggggatgacacggaccaacatgatccaagacagactgccggc

SEQ ID NO: 198 - DNA, 237 bp, Canis familiaris
  source 1..237: mol_type = genomic DNA
ctcccactaactagcaggtatacatagttaaatttctctaacacagagcaatactaccttccacaccagaaaatggcaaaggctaaatataaccacagatctcaaggctactgaactacaygcaggtaatagattatatttaaaacatatcagatgaatctgcactaatactgggggcctataaaactttctaacatacagtagtataagcaggatttccaatcagtgagaaaagga

SEQ ID NO: 199 - DNA, 121 bp, Canis familiaris
  source 1..121: mol_type = genomic DNA
atgtgtaatttacaaagagttcatatattactttatcagttaagcttttgtaattccatamtctatactaattttaaagaggagtgattccttcttgcaattagtttattgcctccgtatg

SEQ ID NO: 200 - DNA, 237 bp, Canis familiaris
  source 1..237: mol_type = genomic DNA
atatatcattccacctatagtaattttcactaatctgcccatttattccctagtgcatacccttaatataaatctgcaacaagaatataacttttctaaaaaaaaaaaaaaagtgtacatrcattagtgatgtgtgtgaccaactaaataccagtgtataagcccatgcccatatttcattttcacgaattatgtttgctgcataaataagacttgtagctttttaaacttacctct

SEQ ID NO: 201 - DNA, 237 bp, Canis familiaris
  source 1..237: mol_type = genomic DNA
gtgtcagtatgttaagccactagtgcactgttaactgctgccatgactaagaaaaaacacagaagctgctgctgctactatgtcactcttgtcatttttaaggtgaatcctcatatgaatragagggagtacatgcttaatggtcagagtgacagcttttgcttcatggcgagccatcgaaaccccacaaatctctttgccccaacagattcttcacctttcttctccagaaatgaa

SEQ ID NO: 202 - DNA, 237 bp, Canis familiaris
  source 1..237: mol_type = genomic DNA
ttatggatcttacaatctagtgattgaaacacaaattagatttgggcttgtctataaaactgggatattttctgatattggaatgaatactgggacagtcccttaattatggtttcatgartgattagtcttatgatacatagtttatgtgtaattgctatttctaatccaaaataaattggacctttcgtttagattaaacatggagtctttgatgtaaataccgtagaaggagtc

SEQ ID NO: 203 - DNA, 237 bp, Canis familiaris
  source 1..237: mol_type = genomic DNA
tgctgtctaaacaggagcttgaaggatgagtaggaagagatttcagatagaacagctgtgctggagcaaagagggtctgagggagcatggtatatttagtggacggcagctagttgcctgscactggagcatggcgggtggggagtaagaggtgggagagaaaactcaatgacaggcagaagccagaccatgaagggcctcacatcctgtgcagaggagttttgatttttatctcct

SEQ ID NO: 204 - DNA, 237 bp, Canis familiaris
  source 1..237: mol_type = genomic DNA
tttgtccttgaaagaagtttttctctttctttcccattttctttttcttcctatttgcttaattatctgttgccagataattcacacctaagttcatagaggaccaatgtcacagatattytcttaaacaaaactggctttgtaacaataaaatttgtctgtttaaaatgtaactaatatcggagatatttacctaaggaagtatttgtaaatagtatctagaaatgcaagaaaata

SEQ ID NO: 205 - DNA, 237 bp, Canis familiaris
  source 1..237: mol_type = genomic DNA
gccaacgctaagattcatatgtctatttttactcaacaccaaataaaggtaccatttctaatccaagaacttcactctgctgtcttctagcacattggcattttccacaggcatttcttgytttacttgatgtatttttttccagtttttcttaatatgatatctgagaaatttttttgctaagtattgattcaaaaatttaaaattaaggttaaattgtggctaatcagcatactg

SEQ ID NO: 206 - DNA, 236 bp, Canis familiaris
  source 1..236: mol_type = genomic DNA
ttttatcatgccaggaaattcttggaatgtagccactgtctgatatttatggttccataagcatttgactctgaaaagtctctaattctggaaaacggccactgatcagttgttaatgcayagcagtaggaaaaaagtcaccccttaaaaggagagagaggacaaaaggaacagcttgtgaggctaaaagtatgacaagtatgacgtctacctatacaggaagtgtatatgcatct

SEQ ID NO: 207 - DNA, 121 bp, Canis familiaris
  source 1..121: mol_type = genomic DNA
gctaataaaggatcaacctctgggctgcagaataacctaatctattcatacctcagtgacrtcctgaattagaaccgggggctgatgaactccaatgcaccagccaaccaaccagagttag

SEQ ID NO: 208 - DNA, 237 bp, Canis familiaris
  source 1..237: mol_type = genomic DNA
tgaatgactttttcaacccgaattttcatgacatttttgtcatgacatttctcatataacctaccgcatgtaaagcaagatctcctattggattctgtcttattttttgtcatcttccaayggtcttaggcaaatgaagtttaagtagtaagattatatgcctcctcccactttggtgcatgcacacagatgcaggaacatgcttagtaactaatctttgtgggacataggaatgcc

SEQ ID NO: 209 - DNA, 237 bp, Canis familiaris
  source 1..237: mol_type = genomic DNA
gccagctctaatgagtttgtttccaagcggtgcttccagaaattgttagtggttggtagttgcaatgggttttgaaattagaggacatcacagcagagtagaatggtttggaacaggggartatgattaggattaatgagatgaaagaaaattctggctagagggctagaagagccatggaagaaaatatacactaaccctttggagtgttcctccaagtgaagatttgcaacattt

SEQ ID NO: 210 - DNA, 237 bp, Canis familiaris
  source 1..237: mol_type = genomic DNA
acgagaagcaagattgccataccgttcctggtaccgggccatgacgttgaccttcaaaagccctgaaacggctgttttcctggctgctgtgagctgtggaactcaggagtaggtatttccygaaaacatttaacatcccatagcaaaggtgttggaggcgtcgtctccattgtcgtttctcccgggctgtggttggcctttctgcgtgagtgcttctccccgctgcgggctggctct

SEQ ID NO: 211 - DNA, 237 bp, Canis familiaris
  source 1..237: mol_type = genomic DNA
taggaaaaaacatctggcctctgactcggatccagtcatcccagcctcattcacacccacccatcagctctcagagaaccttctgagacttcgataaatagctgagcccttaaaatgacarcattgatttggcatggtttgggcaataacttctggctgctgtgatttttaggttttgaatatttagtttctggaaactctgatagaatgaataactttatatgtttatttaattct

SEQ ID NO: 212 - DNA, 237 bp, Canis familiaris
  source 1..237: mol_type = genomic DNA
gtctactgaagccagacagttggttcattagattaattaaagtgcaaactaaccccaatctggtgttttgataacggccacagggctcttgaagttggaatcggccagcatttgacagtgytctcattaaagccacagtggaattgcctctatggtttctcctaaacttttgaatttaccttataacaaagaagtggactttgagcatccctgattgttttttcagtgttaactgct

SEQ ID NO: 213 - DNA, 237 bp, Canis familiaris
  source 1..237: mol_type = genomic DNA
tgttgctttcctgcacacaagcagttgaaccagagtagggaggaatcatttttaggaatgtgttattattattttttaggaatgcacaaaacccatgccaaaaagcccatccacgtctaaygtccttgaacctctccttcactaccaattgtattcttttatgttcccaatcaactggctggcctgaaatagatttctcctaccaagaaatgtagataaaaatatttatttctggaa

SEQ ID NO: 214 - DNA, 237 bp, Canis familiaris
  source 1..237: mol_type = genomic DNA
gtctcagccctctattccagaaggtaggactggccctgggcctgtctacgaggtggtggctgcgagccctcaaggcctggcattgtcaaagttctgacaaccttccccacctatggcagckcagtgttagacgctccaggctgagggttgatgcacactttttcggcttccaaagtgtggccttctcctcagggcttcccatggggtccacaggctggcagcaacctcttggagaaa

SEQ ID NO: 215 - DNA, 237 bp, Canis familiaris
  source 1..237: mol_type = genomic DNA
cagctgtgtcatggaaatggcactttaaaaattcatatgaatcttaacagtaaagcacaagactttggagatatttctcctgttgaatagctgcttggggatgtgccacagatctgtagargtcagcattcactctaagttcccgggaaccatgagacagcagcaaccatggccaccacagcaacacagcaggtgcccataagcccattttacagatggagaaattgggtccagaga

SEQ ID NO: 216 - DNA, 237 bp, Canis familiaris
  source 1..237: mol_type = genomic DNA
cctctggctccccagaacctcagagcttaggggatgtagtggttgtaatcctggatccctctgtggggtggcaggtctggagtggtgagctactgtgagggaactggggtaactgtgaccygagaagaaaggagcgagggagtgagtgtgtgtctgtgaaatatgcctctgtgtgtataaacagggctggagggctcagtgccccccactcccaaagatccacctgttacatccccg

SEQ ID NO: 217 - DNA, 237 bp, Canis familiaris
  source 1..237: mol_type = genomic DNA
ttcttctcttgtgactggtcactaaagacagagatttcaggagagctgactttggtaggaattctcacccttttctggcctaggcctataatttttataccgacagctggagtcccagatrgaagagaccttaaactctttggactatgaagaacctgttttttctctctctctcttttttttccccttaaaacaaaaatttattttcctcaggcctcatcctgtacccagtcttgt

SEQ ID NO: 218 - DNA, 237 bp, Canis familiaris
  source 1..237: mol_type = genomic DNA
agctccaatttagtcatatactaaagaatcaggtcatactctaggcagactctaggcagttagcacatgaaaccagttcacatgctttatcatcatcctttttgttctcaaaacagccaamaacagttctgtataagatatttcacatgtttaattctttcagttcttctagcaagcaggaagcttagaacaagattttagtatttggtttagataacaattgcaaataggagcacc

SEQ ID NO: 219 - DNA, 237 bp, Canis familiaris
  source 1..237: mol_type = genomic DNA
gacttttctagagagaccatggaagatgcatgtggggcctgcccaggctgccacaggggaaaggagccgggaggagggagctgtcaggccacttcctctgatggcccctcagcagcaggargagagcatttcctcaccagatcccactcaacactggccacggtccccctgtggacttcagaactgactcagaactaacctgactgactgcgtatgatttgtctttttaggaggacc

SEQ ID NO: 220 - DNA, 237 bp, Canis familiaris
  source 1..237: mol_type = genomic DNA
cccgcgccaggccggtcctctcctcccagctcctcctctcccgctcgcagtcagggcagccagggaggggagaaattctcatctcaaaactagtaagacaaggccccgcagcgggtctgcrgcgcggaggcggctgcctctcctggtccatactggacacagctgaccacatttcaacaggtaagaatcattttaaatattacccttaaaccaaaaaaagttcttcttttgcttcta

SEQ ID NO: 221 - DNA, 237 bp, Canis familiaris
  source 1..237: mol_type = genomic DNA
cagtattccgattcttctatttgctaattttaaagtgcagatctaagaggacaaccttattattatttccatggtcttagagatcatcttactgttgccccacaatgtccatgcttcccgkgaaagatgtgtgtatccagactcaaagtgaatctaatagggaaggaagactgagaattctattagtaagcaacccgtatttaacaacatggcccagtttgaagatttgcagaaaca

SEQ ID NO: 222 - DNA, 237 bp, Canis familiaris
  source 1..237: mol_type = genomic DNA
tcaggagtgagcctgtacgttatcctgactactgattcccttgcaccaaaaaagcaacgggagcataagggcaagatatgacctttagctaaagggttgcaagttatattactagtcgtcrctgctcaaacacccagcaccagaccctgcatagaatacagaaaagagtcctcaccatcaagccactaccacctgaagcatgaaggagagaacaaggagagatcacctcctaagtgt

SEQ ID NO: 223 - DNA, 237 bp, Canis familiaris
  source 1..237: mol_type = genomic DNA
ctgacctctgctctagtcaattgctctgaaagtacagtcctctgatcctagactcgaaccctctcaagcataacagttccatctactattcactaatccatttatttaactgggagtgttstatgctttggctctgggatatgaaggaaaggacattgtgcccgaacatataggaaagttattgtttaaggagatatacagggaaataattttaaaacaccatggtaatcttttcct

SEQ ID NO: 224 - DNA, 237 bp, Canis familiaris
  source 1..237: mol_type = genomic DNA
cgttttccttataaatttttagaaaacagaacaggaaaaaaaaaaaaagaaagaaaacagaacagagaacaaaccaacatgtcttgatgcctccaggaaccagttttctcatagccttagrggaaacaatttacaaaatatctgaaaagcctgcagatatcttagatccaagattccaaggcataaaaatgtaagtgatcatgtactacgtattactgaaatacagaaagcaaccaa

SEQ ID NO: 225 - DNA, 237 bp, Canis familiaris
  source 1..237: mol_type = genomic DNA
agcaccttgagaatggtgtagtggaaagaaagttgacttttagtaactatgcatttgtctcgttaatgcagtttctcacctgctttgagataatgggaaatggaactaacaggtagtggtracacagatgatggacaatataaagatttgagatatatataaaaaaaatttgatcattatatgtacactttgctagttttgctctacattttttatccacacaaaaagtaatttgca

SEQ ID NO: 226 - DNA, 237 bp, Canis familiaris
  source 1..237: mol_type = genomic DNA
taagtagcctttagtgcaaggaaaagaaaaaggcagtaaggatgaacctttgtttcaaaggtattaggagtcatttaaggaatttcaaaaaaaaaaaaaagaagtgacatgattttgaacraagaagtgactgtcagtactataaagagcacattgcctcaaggagaaactgaagttagagaagccaaattggctgataaaaatctaggccggagatgcaaacacctaaatgaaaac

SEQ ID NO: 227 - DNA, 20 bp, synthetic construct
  misc_feature 1..20: note = Primer
  source 1..20: mol_type = other DNA
gttaccctgcagctgagagt

SEQ ID NO: 228 - DNA, 20 bp, synthetic construct
  misc_feature 1..20: note = Primer
  source 1..20: mol_type = other DNA
atggcgagcatcacagtatc

SEQ ID NO: 229 - DNA, 37 bp, synthetic construct
  misc_feature 1..37: note = Primer
  source 1..37: mol_type = other DNA
gttttcccagtcacgacgttaccctgcagctgagagt

SEQ ID NO: 230 - DNA, 17 bp, synthetic construct
  misc_feature 1..17: note = Primer
  source 1..17: mol_type = other DNA
gttttcccagtcacgac

SEQ ID NO: 231 - DNA, 19 bp, synthetic construct
  misc_feature 1..19: note = Primer
  source 1..19: mol_type = other DNA
gttaccctgcagctgagag

SEQ ID NO: 232 - DNA, 20 bp, synthetic construct
  misc_feature 1..20: note = Primer
  source 1..20: mol_type = other DNA
agggtcgtactgtacttggg

SEQ ID NO: 233 - DNA, 21 bp, synthetic construct
  misc_feature 1..21: note = Primer
  source 1..21: mol_type = other DNA
cgtctggatgggaagtttctc

SEQ ID NO: 234 - DNA, 19 bp, synthetic construct
  misc_feature 1..19: note = Primer
  source 1..19: mol_type = other DNA
ttgtcggacttcagggagg

SEQ ID NO: 235 - DNA, 20 bp, synthetic construct
  misc_feature 1..20: note = Primer
  source 1..20: mol_type = other DNA
ccggcggtgggactccccgc

SEQ ID NO: 236 - DNA, 989 bp, Canis familiaris
  source 1..989: mol_type = genomic DNA
tcagcacccaggaggcagtcatcacttaccagccttatcttattcaaccccaggacctcagggaccatgtaaacgacatggggtttgaagctgtcatcaagaacagagtggcacccgtaagcctgggacccattgatattgggcggttacagaggaccaacccaaagatgcctttgacttctgataaccagaatctcaataactctgagaccttgggccatcaagggagccatgtggttaccctgcagctgagagtcgacggaatgcactgtcagtcttgtgtcctgaacattgaagagaatataggccaactccccggggttcagaatgtgcaagtgtccttggagaacagaacggcccaagtacagtacgacccttcttgtgtcaccgcaggggccctgcagagggccattgaagctctcccaccagggaactttaaagtttctcttcctgccgcagcagcaggaagtgagacaggtaacaggttttcggcatgtgccgcccccgccccaagaaccccggcaccgggcaggtgcgatactgtgatgctcgccattgtgggcatgacctgtgcatcctgcgtccagtcgatcgaaggcctgatctcccagagggaaggggtgcagcaaatatctgtctctctggctgaagggaccgcagtggttctctatgatccctctataattggcccggaagaactccgagctgccgtcgaggagatgggatttgagacttcagtcctctctggtatgtagtggcaccccgggtcttctcctctctccttgggccttacggcagagtgcctgcagggtggcacaggggagccaccccagctgctcgcctgtcgggttggccaagtcccgcagcgtttccctgtgtgttgaatgtgtccgggtgggagaaagagaactttctggtgtgtagattttgcctctcatggggctgggactacattgctaaattctttgttgttgttattttttttaact

SEQ ID NO: 237 - DNA, 995 bp, Canis familiaris
  source 1..995: mol_type = genomic DNA
tcagcacccaggaggcagtcatcacttaccagccttatcttattcaaccccaggacctcagggaccatgtaaacgacatggggtttgaagctgtcatcaagaacagagtggcacccgtaagcctgggacccattgatattgggcggttacagaggaccaacccaaagatgcctttgacttctgataaccagaatctcaataactctgagaccttgggccatcaagggagccatgtggttaccctgcagctgagagtcgacggaatgcactgtcagtcttgtgtcctgaacattgaagagaatataggccaactccccggggttcagaatgtgcaagtgtccttggagaacagaacggcccaagtacagtacgacccttcttgtgtcaccgcaggggccctgcagagggccattgaagctctcccaccagggaactttaaagtttctcttcctgccgcagcagcaggaagtgagacaggtaacaggttttcggcatgtgccgcccccgcccccgccccaagaaccccggcaccgggcaggtgcgatactgtgatgctcgccattgtgggcatgacctgtgcatcctgcgtccagtcgatcgaaggcctgatctcccagagggaaggggtgcagcaaatatctgtctctctggctgaagggaccgcagtggttctctatgatccctctataattggcccggaagaactccgagctgccgtcgaggagatgggatttgagacttcagtcctctctggtatgtagtggcaccccgggtcttctcctctctccttgggccttacggcagagtgcctgcagggtggcacaggggagccaccccagctgctcgcctgtcgggttggccaagtcccgcagcgtttccctgtgtgttgaatgtgtccgggtgggagaaagagaactttctggtgtgtagattttgcctctcatggggctgggactacattgctaaattctttgttgttgttattttttttaact

SEQ ID NO: 238 - DNA, 1001 bp, Canis familiaris
  source 1..1001: mol_type = genomic DNA
tcagcacccaggaggcagtcatcacttaccagccttatcttattcaaccccaggacctcagggaccatgtaaacgacatggggtttgaagctgtcatcaagaacagagtggcacccgtaagcctgggacccattgatattgggcggttacagaggaccaacccaaagatgcctttgacttctgataaccagaatctcaataactctgagaccttgggccatcaagggagccatgtggttaccctgcagctgagagtcgacggaatgcactgtcagtcttgtgtcctgaacattgaagagaatataggccaactccccggggttcagaatgtgcaagtgtccttggagaacagaacggcccaagtacagtacgacccttcttgtgtcaccgcaggggccctgcagagggccattgaagctctcccaccagggaactttaaagtttctcttcctgccgcagcagcaggaagtgagacaggtaacaggttttcggcatgtgccgcccccgcccccgcccccgccccaagaaccccggcaccgggcaggtgcgatactgtgatgctcgccattgtgggcatgacctgtgcatcctgcgtccagtcgatcgaaggcctgatctcccagagggaaggggtgcagcaaatatctgtctctctggctgaagggaccgcagtggttctctatgatccctctataattggcccggaagaactccgagctgccgtcgaggagatgggatttgagacttcagtcctctctggtatgtagtggcaccccgggtcttctcctctctccttgggccttacggcagagtgcctgcagggtggcacaggggagccaccccagctgctcgcctgtcgggttggccaagtcccgcagcgtttccctgtgtgttgaatgtgtccgggtgggagaaagagaactttctggtgtgtagattttgcctctcatggggctgggactacattgctaaattctttgttgttgttattttttttaact

SEQ ID NO: 239 - DNA, 33 bp, synthetic construct
  source 1..33: mol_type = other DNA
tgtgccgcccccgcccccgcccccgccccaaga

SEQ ID NO: 240 - protein, 11 aa, synthetic construct
CAAPAPAPAPR

SEQ ID NO: 241 - DNA, 27 bp, synthetic construct
  source 1..27: mol_type = other DNA
tgtgccgcccccgcccccgccccaaga

SEQ ID NO: 242 - DNA, 21 bp, synthetic construct
  source 1..21: mol_type = other DNA
tgtgccgcccccgccccaaga

SEQ ID NO: 243 - DNA, 15 bp, synthetic construct
  source 1..15: mol_type = other DNA
tccccgcgggccacg

SEQ ID NO: 244 - DNA, 15 bp, synthetic construct
  source 1..15: mol_type = other DNA
tccccgcaggccacg

SEQ ID NO: 245 - protein, 5 aa, synthetic construct
SPRAT

SEQ ID NO: 246 - protein, 5 aa, synthetic construct
SPQAT